European Patent Specification EP 4 499 871 B1, published September 23, 2026. Title: METHODS FOR CHEMICAL CLEAVAGE OF SURFACE-BOUND POLYNUCLEOTIDES. Applicant: Illumina Cambridge Limited. Application WO. The sequence listing filed with the application follows.

SEQUENCE LISTING (25 sequences)

SEQ ID NO: 1 - DNA, 29 bp, synthetic construct
  source 1..29: mol_type = other DNA
  misc_feature 23: note = n is a deoxyuridine
aatgatacggcgaccaccgaganctacac

SEQ ID NO: 2 - DNA, 24 bp, synthetic construct
  source 1..24: mol_type = other DNA
  misc_feature 22: note = n is a 8-oxo-guanine
caagcagaagacggcatacganat

SEQ ID NO: 3 - DNA, 39 bp, synthetic construct
  misc_feature 1: note = 5 prime alkyne
  source 1..39: mol_type = other DNA
  misc_feature 33: note = n is a deoxyuridine
ttttttttttaatgatacggcgaccaccgaganctacac

SEQ ID NO: 4 - DNA, 34 bp, synthetic construct
  misc_feature 32: note = n is a 8-oxo-guanine
  misc_feature 1: note = 5 prime alkyne
  source 1..34: mol_type = other DNA
ttttttttttcaagcagaagacggcatacganat

SEQ ID NO: 5 - DNA, 20 bp, synthetic construct
  source 1..20: mol_type = other DNA
aatgatacggcgaccaccga

SEQ ID NO: 6 - DNA, 21 bp, synthetic construct
  source 1..21: mol_type = other DNA
caagcagaagacggcatacga

SEQ ID NO: 7 - DNA, 29 bp, synthetic construct
  misc_feature 23: note = n is a vinyl substituted T nucleoside
  source 1..29: mol_type = other DNA
aatgatacggcgaccaccgaganctacac

SEQ ID NO: 8 - DNA, 27 bp, synthetic construct
  misc_feature 1..3: note = diol linker subject to chemical cleavage
  source 1..27: mol_type = other DNA
nnncaagcagaagacggcatacgagat

SEQ ID NO: 9 - DNA, 35 bp, synthetic construct
  misc_feature 29: note = a vinyl substituted T nucleoside
  misc_feature 1: note = 5 prime alkyne
  source 1..35: mol_type = other DNA
ttttttaatgatacggcgaccaccgaganctacac

SEQ ID NO: 10 - DNA, 33 bp, synthetic construct
  misc_feature 7..9: note = diol linker subject to chemical cleavage
  misc_feature 1: note = 5 prime alkyne
  source 1..33: mol_type = other DNA
ttttttnnncaagcagaagacggcatacgagat

SEQ ID NO: 11 - DNA, 33 bp, synthetic construct
  misc_feature 2..4: note = diol linker subject to chemical cleavage
  misc_feature 1: note = 5 prime alkyne
  source 1..33: mol_type = other DNA
tnnntttttcaagcagaagacggcatacgagat

SEQ ID NO: 12 - DNA, 32 bp, synthetic construct
  misc_feature 2..3: note = diol linker subject to chemical cleavage
  misc_feature 1: note = 5 prime alkyne
  source 1..32: mol_type = other DNA
tnntttttcaagcagaagacggcatacgagat

SEQ ID NO: 13 - DNA, 31 bp, synthetic construct
  misc_feature 2: note = diol linker subject to chemical cleavage
  misc_feature 1: note = 5 prime alkyne
  source 1..31: mol_type = other DNA
tntttttcaagcagaagacggcatacgagat

SEQ ID NO: 14 - DNA, 33 bp, synthetic construct
  misc_feature 1..3: note = diol linker subject to chemical cleavage
  misc_feature 1: note = Alkyne on terminal end
  source 1..33: mol_type = other DNA
nnnttttttcaagcagaagacggcatacgagat

SEQ ID NO: 15 - DNA, 32 bp, synthetic construct
  misc_feature 1..2: note = diol linker subject to chemical cleavage
  misc_feature 1: note = Alkyne on terminal end
  source 1..32: mol_type = other DNA
nnttttttcaagcagaagacggcatacgagat

SEQ ID NO: 16 - DNA, 31 bp, synthetic construct
  misc_feature 1: note = diol linker subject to chemical cleavage
  misc_feature 1: note = Alkyne on terminal end
  source 1..31: mol_type = other DNA
nttttttcaagcagaagacggcatacgagat

SEQ ID NO: 17 - DNA, 33 bp, synthetic construct
  misc_feature 3..5: note = diol linker subject to chemical cleavage
  misc_feature 1: note = 5 prime alkyne
  source 1..33: mol_type = other DNA
ttnnnttttcaagcagaagacggcatacgagat

SEQ ID NO: 18 - DNA, 32 bp, synthetic construct
  misc_feature 3..4: note = diol linker subject to chemical cleavage
  misc_feature 1: note = 5 prime alkyne
  source 1..32: mol_type = other DNA
ttnnttttcaagcagaagacggcatacgagat

SEQ ID NO: 19 - DNA, 31 bp, synthetic construct
  misc_feature 3: note = diol linker subject to chemical cleavage
  misc_feature 1: note = 5 prime alkyne
  source 1..31: mol_type = other DNA
ttnttttcaagcagaagacggcatacgagat

SEQ ID NO: 20 - DNA, 33 bp, synthetic construct
  misc_feature 4..6: note = diol linker subject to chemical cleavage
  misc_feature 1: note = 5 prime alkyne
  source 1..33: mol_type = other DNA
tttnnntttcaagcagaagacggcatacgagat

SEQ ID NO: 21 - DNA, 32 bp, synthetic construct
  misc_feature 4..5: note = diol linker subject to chemical cleavage
  misc_feature 1: note = 5 prime alkyne
  source 1..32: mol_type = other DNA
tttnntttcaagcagaagacggcatacgagat

SEQ ID NO: 22 - DNA, 31 bp, synthetic construct
  misc_feature 4: note = diol linker subject to chemical cleavage
  misc_feature 1: note = 5 prime alkyne
  source 1..31: mol_type = other DNA
tttntttcaagcagaagacggcatacgagat

SEQ ID NO: 23 - DNA, 33 bp, synthetic construct
  misc_feature 5..7: note = diol linker subject to chemical cleavage
  misc_feature 1: note = 5 prime alkyne
  source 1..33: mol_type = other DNA
ttttnnnttcaagcagaagacggcatacgagat

SEQ ID NO: 24 - DNA, 32 bp, synthetic construct
  misc_feature 5..6: note = diol linker subject to chemical cleavage
  misc_feature 1: note = 5 prime alkyne
  source 1..32: mol_type = other DNA
ttttnnttcaagcagaagacggcatacgagat

SEQ ID NO: 25 - DNA, 31 bp, synthetic construct
  misc_feature 5: note = diol linker subject to chemical cleavage
  misc_feature 1: note = 5 primer alkyne
  source 1..31: mol_type = other DNA
ttttnttcaagcagaagacggcatacgagat